European Patent Application EP 4 332 114 A1, published March 6, 2024. Title: METHOD FOR SCREENING alphabeta-TCR HETERODIMER MUTANTS. Applicant: LIYANG TCR BIOTHERAPEUTICS CO. LTD. Application PCT/CN2021/091681. The sequence listing filed with the application follows.

SEQUENCE LISTING (53 sequences)

SEQ ID NO: 1 - protein, 37 aa, Artificial Sequence
  A1 peptide
STTVAQLEEKVKTLRAQNYELKSRVQRLREQVAQLAS

SEQ ID NO: 2 - protein, 37 aa, Artificial Sequence
  B1 peptide
STSVDELQAEVDQLQDENYALKTKVAQLRKKVEKLSE

SEQ ID NO: 3 - protein, 8 aa, Artificial Sequence
  linker
GGSGGGGG

SEQ ID NO: 4 - protein, 130 aa, Artificial Sequence
  ݶ chain constant region
EDLNKVFPPEVAVFEPSEAEISHTQKATLVCLATGFFPDHVELSWWVNGKEVHSGVSTDPQPLKEQPALNDSRYCLSSRLRVSATFWQNPRNHFRCQVQFYGLSENDEWTQDRAKPVTQIVSAEAWGRAD

SEQ ID NO: 5 - protein, 93 aa, Artificial Sequence
  ݵ chain constant region
IQNPDPAVYQLRDSKSSDKSVCLFTDFDSQTNVSQSKDSDVYITDKTVLDMRSMDFKSNSAVAWSNKSDFACANAFNNSIIPEDTFFPSPESS

SEQ ID NO: 6 - protein, 130 aa, Artificial Sequence
  ݶ chain constant region
EDLKNVFPPEVAVFEPSEAEISHTQKATLVCLATGFYPDHVELSWWVNGKEVHSGVSTDPQPLKEQPALNDSRYCLSSRLRVSATFWQNPRNHFRCQVQFYGLSENDEWTQDRAKPVTQIVSAEAWGRAD

SEQ ID NO: 7 - DNA, 23 bp, Artificial Sequence
  ribosomal binding site
tttgtttaactttaagaaggaga

SEQ ID NO: 8 - DNA, 486 bp, Artificial Sequence
  Skp gene
atgaaaaagtggttattagctgcaggtctcggtttagcactggcaacttctgctcaggcggctgacaaaattgcaatcgtcaacatgggcagcctgttccagcaggtagcgcagaaaaccggtgtttctaacacgctggaaaatgagttcaaaggccgtgccagcgaactgcagcgtatggaaaccgatctgcaggctaaaatgaaaaagctgcagtccatgaaagcgggcagcgatcgcactaagctggaaaaagacgtgatggctcagcgccagacttttgctcagaaagcgcaggcttttgagcaggatcgcgcacgtcgttccaacgaagaacgcggcaaactggttactcgtatccagactgctgtgaaatccgttgccaacagccaggatatcgatctggttgttgatgcaaacgccgttgcttacaacagcagcgatgtaaaagacatcactgccgacgtactgaaacaggttaaataa

SEQ ID NO: 9 - DNA, 894 bp, Artificial Sequence
  between the signal peptide and the Amber Stop Codon
atgaaatacctattgcctacggcagccgctggattgttattactcgcggcccagccggccatggctctaatagtgactaatagtgactaatagtgagtgagcaagggcgaggagctgttcaccggggtggtgcccatcctggtcgagctggacggcgacgtaaacggccacaagttcagcgtgtccggcgagggcgagggcgatgccacctacggcaagctgaccctgaagttcatctgcaccaccggcaagctgcccgtgccctggcccaccctcgtgaccaccctgacctacggcgtgcagtgcttcagccgctaccccgaccacatgaagcagcacgacttcttcaagtccgccatgcccgaaggctacgtccaggagcgcaccatcttcttcaaggacgacggcaactacaagacccgcgccgaggtgaagttcgagggcgacaccctggtgaaccgcatcgagctgaagggcatcgacttcaaggaggacggcaacatcctggggcacaagctggagtacaactacaacagccacaacgtctatatcatggccgacaagcagaagaacggcatcaaggtgaacttcaagatccgccacaacatcgaggacggcagcgtgcagctcgccgaccactaccagcagaacacccccatcggcgacggccccgtgctgctgcccgacaaccactacctgagcacccagtccgccctgagcaaagaccccaacgagaagcgcgatcacatggtcctgctggagttcgtgaccgccgccgggatcactctcggcatggacgagctgtacaagtaatagtgactaatagtgactaatagtgatgcggccgctggatccgaacagaaactgatcagcgaagaggatctggctgaatag

SEQ ID NO: 10 - protein, 113 aa, Artificial Sequence
  wild-type TCR1 ݵ
GQNIDQPTEMTATEGAIVQINCTYQTSGFNGLFWYQQHAGEAPTFLSYNVLDGLEEKGRFSSFLSRSKGYSYLLLKELQMKDSASYLCAVSNSGAGSYQLTFGKGTKLSVIPN

SEQ ID NO: 11 - protein, 114 aa, Artificial Sequence
  wild-type TCR1 ݶ
DTGVSQDPRHKITKRGQNVTFRCDPISEHNRLYWYRQTLGQGPEFLTYFQNEAQLEKSRLLSDRFSAERPKGSFSTLEIQRTEQGDSAMYLCASSLGLGEETQYFGPGTRLLVL

SEQ ID NO: 12 - protein, 109 aa, Artificial Sequence
  wild-tpye TCR2 ݵ
ELKVEQNPLFLSMQEGKNYTIYCNYSTTSDRLYWYRQDPGKSLESLFVLLSNGAVKQEGRLMASLDTKARLSTLHITAAVHDLSATYFCGGGADGLTFGKGTHLIIQPY

SEQ ID NO: 13 - protein, 114 aa, Artificial Sequence
  wild-tpye TCR2 ݶ
DTGVSQDPRHKITKRGQNVTFRCDPISEHNRLYWYRQTLGQGPEFLTYFQNEAQLEKSRLLSDRFSAERPKGSFSTLEIQRTEQGDSAMYLCASSLYGGGDTQYFGPGTRLTVL

SEQ ID NO: 14 - protein, 110 aa, Artificial Sequence
  wild-type TCR3 ݵ
GIQVEQSPPDLILQEGANSTLRCNFSDSVNNLQWFHQNPWGQLINLFYIPSGTKQNGRLSATTVATERYSLLYISSSQTTDSGVYFCAVEGDSNYQLIWGAGTKLIIKPD

SEQ ID NO: 15 - protein, 112 aa, Artificial Sequence
  wild-type TCR3 ݶ
DTGVSQDPRHKITKRGQNVTFRCDPISEHNRLYWYRQTLGQGPEFLTYFQNEAQLEKSRLLSDRFSAERPKGSFSTLEIQRTEQGDSAMYLCASRHLYNEQFFGPGTRLTVL

SEQ ID NO: 16 - protein, 117 aa, Artificial Sequence
  wild-type TCR4 ݵ
AQKITQTQPGMFVQEKEAVTLDCTYDTSDQSYGLFWYKQPSSGEMIFLIYQGSYDEQNATEGRYSLNFQKARKSANLVISASQLGDSAMYFCAMREPRGSARQLTFGSGTQLTVLPD

SEQ ID NO: 17 - protein, 117 aa, Artificial Sequence
  wild-type TCR4 ݶ
DGGITQSPKYLFRKEGQNVTLSCEQNLNHDAMYWYRQDPGQGLRLIYYSQIVNDFQKGDIAEGYSVSREKKESFPLTVTSAQKNPTAFYLCASSQGIGLAGGIYEQYFGPGTRLTVT

SEQ ID NO: 18 - protein, 13 aa, Artificial Sequence
  TCR1 CDR3 A0
AVSNSGAGSYQLT

SEQ ID NO: 19 - protein, 13 aa, Artificial Sequence
  TCR1 CDR3 A1
AVSNSLDGYYQLT

SEQ ID NO: 20 - protein, 12 aa, Artificial Sequence
  TCR1 CDR3 B0
ASSLGLGEETQY

SEQ ID NO: 21 - protein, 12 aa, Artificial Sequence
  TCR1 CDR3 B1
ASSLGYGRETQY

SEQ ID NO: 22 - protein, 12 aa, Artificial Sequence
  TCR1 CDR3 B2
ASSLGFGRETQY

SEQ ID NO: 23 - protein, 12 aa, Artificial Sequence
  TCR1 CDR3 B3
ASSLGYGTETQY

SEQ ID NO: 24 - protein, 12 aa, Artificial Sequence
  TCR1 CDR3 B4
ASSLGYGQETQY

SEQ ID NO: 25 - protein, 10 aa, Artificial Sequence
  TR3 CDR3 B0
ASRHLYNEQF

SEQ ID NO: 26 - protein, 10 aa, Artificial Sequence
  TCR3 CDR3 B1
ASQSWYNEQF

SEQ ID NO: 27 - protein, 10 aa, Artificial Sequence
  TCR3 CDR3 B2
ASQRWYNEQF

SEQ ID NO: 28 - protein, 10 aa, Artificial Sequence
  TCR3 CDR3 B3
ASRREFNEQF

SEQ ID NO: 29 - protein, 10 aa, Artificial Sequence
  TCR3 CDR3 B4
ASRHEFDEQF

SEQ ID NO: 30 - protein, 10 aa, Artificial Sequence
  TCR3 CDR3 B5
ASRLLFNEQF

SEQ ID NO: 31 - protein, 16 aa, Artificial Sequence
  TCR4 CDR3 B0
ASSQGIGLAGGIYEQY

SEQ ID NO: 32 - protein, 16 aa, Artificial Sequence
  TCR4 CDR3 B1
ASSLTIGLAGGIYEQY

SEQ ID NO: 33 - protein, 16 aa, Artificial Sequence
  TCR4 CDR3 B2
ASSLTRGLAGGIYEQY

SEQ ID NO: 34 - protein, 16 aa, Artificial Sequence
  TCR4 CDR3 B3
ASSLTSGLAGGIYEQY

SEQ ID NO: 35 - protein, 16 aa, Artificial Sequence
  TCR4 CDR3 B4
ASALTWGLAGGIYEQY

SEQ ID NO: 36 - protein, 16 aa, Artificial Sequence
  TCR4 CDR3 B5
ASSLGIGLAGGIYEQY

SEQ ID NO: 37 - protein, 16 aa, Artificial Sequence
  TCR4 CDR3 B6
ASSQTIGLAGGIYEQY

SEQ ID NO: 38 - protein, 16 aa, Artificial Sequence
  TCR4 CDR3 B7
ASSQGRGLAGGIYEQY

SEQ ID NO: 39 - protein, 16 aa, Artificial Sequence
  TCR4 CDR3 B8
ASSQGSGLAGGIYEQY

SEQ ID NO: 40 - protein, 8 aa, Artificial Sequence
  TCR2-3-ELISA-1
GIGDDGLT

SEQ ID NO: 41 - protein, 8 aa, Artificial Sequence
  TCR2-3-ELISA-2
GAGTDGLT

SEQ ID NO: 42 - protein, 8 aa, Artificial Sequence
  TCR2-3-ELISA-3
GAGVDGLT

SEQ ID NO: 43 - protein, 8 aa, Artificial Sequence
  TCR2-3-ELISA-4
GVGVDGLT

SEQ ID NO: 44 - protein, 8 aa, Artificial Sequence
  TCR2-3-ELISA-5
GVGDDGLT

SEQ ID NO: 45 - protein, 8 aa, Artificial Sequence
  TCR2-3-ELISA-6
AGGVDGLT

SEQ ID NO: 46 - protein, 8 aa, Artificial Sequence
  TCR2-3-ELISA-7
AAGVDGLT

SEQ ID NO: 47 - protein, 8 aa, Artificial Sequence
  TCR2-3-ELISA-8
AAGTDGLT

SEQ ID NO: 48 - protein, 8 aa, Artificial Sequence
  TCR2-3-ELISA-9
AVGDDGLT

SEQ ID NO: 49 - protein, 8 aa, Artificial Sequence
  TCR2-3-ELISA-10
AIGDDGLT

SEQ ID NO: 50 - protein, 8 aa, Artificial Sequence
  TCR2-3-ELISA-11
AEGVDGLT

SEQ ID NO: 51 - protein, 8 aa, Artificial Sequence
  TCR2-3-ELISA-12
SVGDDGLT

SEQ ID NO: 52 - protein, 8 aa, Artificial Sequence
  TCR2-3-ELISA-13
AVGVDGLT

SEQ ID NO: 53 - protein, 8 aa, Artificial Sequence
  TCR2-3-ELISA-14
AVGTDGLT